European Patent Application EP 4 286 510 A1, published December 6, 2023. Title: Oral Coronavirus Vaccine. Applicant: NATIONAL UNIVERSITY CORPORATION KOBE UNIVERSITY KYOTO UNIVERSITY. The sequence listing filed with the application follows.

SEQUENCE LISTING (29 sequences)

SEQ ID NO: 1 - protein, 1273 aa, coronavirus
MFVFLVLLPLVSSQCVNLTTRTQLPPAYTNSFTRGVYYPDKVFRSSVLHSTQDLFLPFFSNVTWFHAIHVSGTNGTKRFDNPVLPFNDGVYFASTEKSNIIRGWIFGTTLDSKTQSLLIVNNATNVVIKVCEFQFCNDPFLGVYYHKNNKSWMESEFRVYSSANNCTFEYVSQPFLMDLEGKQGNFKNLREFVFKNIDGYFKIYSKHTPINLVRDLPQGFSALEPLVDLPIGINITRFQTLLALHRSYLTPGDSSSGWTAGAAAYYVGYLQPRTFLLKYNENGTITDAVDCALDPLSETKCTLKSFTVEKGIYQTSNFRVQPTESIVRFPNITNLCPFGEVFNATRFASVYAWNRKRISNCVADYSVLYNSASFSTFKCYGVSPTKLNDLCFTNVYADSFVIRGDEVRQIAPGQTGKIADYNYKLPDDFTGCVIAWNSNNLDSKVGGNYNYLYRLFRKSNLKPFERDISTEIYQAGSTPCNGVEGFNCYFPLQSYGFQPTNGVGYQPYRVVVLSFELLHAPATVCGPKKSTNLVKNKCVNFNFNGLTGTGVLTESNKKFLPFQQFGRDIADTTDAVRDPQTLEILDITPCSFGGVSVITPGTNTSNQVAVLYQDVNCTEVPVAIHADQLTPTWRVYSTGSNVFQTRAGCLIGAEHVNNSYECDIPIGAGICASYQTQTNSPRRARSVASQSIIAYTMSLGAENSVAYSNNSIAIPTNFTISVTTEILPVSMTKTSVDCTMYICGDSTECSNLLLQYGSFCTQLNRALTGIAVEQDKNTQEVFAQVKQIYKTPPIKDFGGFNFSQILPDPSKPSKRSFIEDLLFNKVTLADAGFIKQYGDCLGDIAARDLICAQKFNGLTVLPPLLTDEMIAQYTSALLAGTITSGWTFGAGAALQIPFAMQMAYRFNGIGVTQNVLYENQKLIANQFNSAIGKIQDSLSSTASALGKLQDVVNQNAQALNTLVKQLSSNFGAISSVLNDILSRLDKVEAEVQIDRLITGRLQSLQTYVTQQLIRAAEIRASANLAATKMSECVLGQSKRVDFCGKGYHLMSFPQSAPHGVVFLHVTYVPAQEKNFTTAPAICHDGKAHFPREGVFVSNGTHWFVTQRNFYEPQIITTDNTFVSGNCDVVIGIVNNTVYDPLQPELDSFKEELDKYFKNHTSPDVDLGDISGINASVVNIQKEIDRLNEVAKNLNESLIDLQELGKYEQYIKWPWYIWLGFIAGLIAIVMVTIMLCCMTSCCSCLKGCCSCGSCCKFDEDDSEPVLKGVKLHYT

SEQ ID NO: 2 - protein, 195 aa, coronavirus
ITNLCPFGEVFNATRFASVYAWNRKRISNCVADYSVLYNSASFSTFKCYGVSPTKLNDLCFTNVYADSFVIRGDEVRQIAPGQTGKIADYNYKLPDDFTGCVIAWNSNNLDSKVGGNYNYLYRLFRKSNLKPFERDISTEIYQAGSTPCNGVEGFNCYFPLQSYGFQPTNGVGYQPYRVVVLSFELLHAPATVCG

SEQ ID NO: 3 - DNA, 2043 bp, coronavirus
atgtttgtcttcctcgtgctgctccccctcgtgtcgtcgcaatgtgtgaatctcacgaccaggacccagctcccgcccgcttacacgaattcgtttacccgcggtgtttactatccggataaggtgttccgtagctcggtcctgcatagcacgcaagacctgtttctcccgtttttctccaacgtgacgtggttccatgcgattcacgtgtcggggacgaacggcacgaagaggttcgacaacccggtcctgccgttcaatgatggcgtttatttcgcgtcgaccgagaagagcaatattatccgtggttggatttttgggacgaccctggactccaaaacgcagtcgctcctcattgttaataatgctaccaacgttgtgatcaaagtttgtgaattccagttctgcaacgatccctttctgggggtctattaccataagaataacaaatcgtggatggaatcggagtttcgcgtgtatagctcggctaataattgtacgttcgaatatgtcagccaaccctttctgatggatctcgaaggtaaacaaggtaacttcaaaaatctccgtgaattcgtttttaagaacattgatggttactttaagatttattcgaagcatacccccattaatctcgtgcgggacctcccgcaaggattcagcgccctcgagcccctggttgatctcccgatcggaattaacatcacccgttttcaaacgctgctggctctccatcgctcctacctgacccccggtgactcgtcctcgggatggacggcgggcgctgcggcgtattacgtggggtacctgcagccgaggacgttcctgctgaagtacaatgagaatggtaccattacggatgctgtcgactgtgctctggaccccctctcggaaacgaagtgcaccctgaagtcctttaccgtcgaaaagggaatctaccaaacgagcaatttcagggtgcaaccgaccgaatcgatcgtgaggtttcccaacatcaccaacctctgccccttcggcgaagtgttcaacgccacgcgctttgcctccgtgtatgcttggaatcgtaaaaggatctccaattgcgtcgctgactattccgttctgtataattccgcctccttttcgacgttcaagtgctatggagttagccccacgaagctcaatgacctgtgcttcaccaacgtttatgcggatagctttgtcatccggggtgacgaagttaggcaaattgcgcccggccaaaccggtaaaatcgctgattacaactataaactgcccgacgatttcaccggttgcgttatcgcctggaattccaacaatctcgattcgaaggtcggaggtaactataactatctgtatcgtctgttccgtaaatccaatctgaaaccctttgaacgggacatttccaccgaaatttatcaagccggatccaccccgtgtaacggggttgaaggtttcaactgctacttcccgctgcaatcgtacggattccagcccaccaatggagtgggatatcaaccgtaccgtgtcgtggtgctgagcttcgaactcctgcacgcgcccgccacggtgtgtggacccaagaaaagcacgaatctcgtgaagaataaatgcgttaattttaacttcaatgggctgaccggaacgggggtcctcacggagtccaataagaaatttctgcccttccaacagtttggtcgggatatcgcggatacgaccgatgcggtccgtgatccgcaaacgctggagattctcgatatcaccccgtgtagctttggaggggtctcggttatcacgcccgggaccaacacctcgaatcaagttgctgttctctaccaagacgtcaattgtacggaggtcccggtggctattcatgccgaccagctgacgcccacctggagggtctactccaccgggtcgaatgtgttccagacgcgtgccggttgcctgattggcgccgagcacgttaataacagctatgaatgtgatatcccgattggagctggaatctgcgcgtcctaccaaacgcaaacgaactccccc

SEQ ID NO: 4 - DNA, 21 bp, Artificial Sequence
  Primer pSC101 End F
tatgcacagatgaaaacggtg

SEQ ID NO: 5 - DNA, 22 bp, Artificial Sequence
  Primer GLBP End R
agtactctcggaaacagacagg

SEQ ID NO: 6 - DNA, 3 bp, Artificial Sequence
  Stop codon
taa

SEQ ID NO: 7 - DNA, 34 bp, Artificial Sequence
  Primer S1-Infusion F
gtttccgagagtactatgtttgtcttcctcgtgc

SEQ ID NO: 8 - DNA, 34 bp, Artificial Sequence
  Primer S1-Infusion R
tttcatctgtgcatattagggggagttcgtttgc

SEQ ID NO: 9 - DNA, 34 bp, Artificial Sequence; identical to SEQ ID NO: 7
  Primer S1AB-Infusion F

SEQ ID NO: 10 - DNA, 33 bp, Artificial Sequence
  Primer S1AB-Infusion R
tttcatctgtgcatattactccagcgtttgcgg

SEQ ID NO: 11 - DNA, 33 bp, Artificial Sequence
  Primer S1B-330-583 Infusion F
gtttccgagagtactcccaacatcaccaacctc

SEQ ID NO: 12 - DNA, 33 bp, Artificial Sequence; identical to SEQ ID NO: 10
  Primer S1B-330-583 Infusion R

SEQ ID NO: 13 - DNA, 28 bp, Artificial Sequence
  Primer S1B-332-526 F
gcactcgagatcaccaacctctgcccct

SEQ ID NO: 14 - DNA, 30 bp, Artificial Sequence
  Primer S1B-332-526 R
ccagcatgcttcatccacacaccgtggcgg

SEQ ID NO: 15 - DNA, 34 bp, Artificial Sequence
  Primer S1B-332-526 Infusion F
ggaaaactgtccatacatatgggcgatggcgagg

SEQ ID NO: 16 - DNA, 36 bp, Artificial Sequence
  Primer S1B-332-526 Infusion R
tttcatctgtgcatagcatgcttcatccacacaccg

SEQ ID NO: 17 - DNA, 27 bp, Artificial Sequence
  Primer S1B-332-526 N501Y F
ttccagcccacctacggagtgggatat

SEQ ID NO: 18 - DNA, 27 bp, Artificial Sequence
  Primer S1B-332-526 N501Y R
atatcccactccgtaggtgggctggaa

SEQ ID NO: 19 - DNA, 2368 bp, Artificial Sequence
  GLBP-S1B-332-526 fusion gene
catatgggcgatggcgaggcgaacgccacggttgacggcacgcacttcaacgtgcgtagcctgtggcagctctaccagttgctgagactgctcgtgtagcgtctcattaaggtgcggtgccccctggtcgggtatcgcgccggcgacctgaaaaccgataatgttggcaagtgcttgcaatttgcggtggacgattgcaagctaacgtcttggattgttgccgctatccaatatctcattaggcctaccggtggaccaaaagtacgttgctttgtaaggggagttaatgaaatgaacaaactcgcacaatcgagcatcgaaccggtttaatgctactcgcctcaacgggacgcgcggtaattgttagctaagttgacaataaaagaatgagggcatacattagtaatcagtcatcacactgagatgatgatttcactacgaaggagtagagatatggtatctcgcaataagcgcatcgtggctgcttttgccgcggtagcagcaatgggaatgggcttggccggttgcggcagcgacactgccggcgacacgaagaccaccgatgatggtggcgtggtcaacatcacctacatgcaccgtctgccggattccgagggcatgactctggtcaacgacatcgttgccaagtggaataagcagcatccggatattcaggtcaaggccaccaagttcgatggtaaggcctctgacatgatcaagaagcttgagaccgacgtcaagtccggcgaggctccggatctggctcaggtcggttacgccgagctgcctgaggtcttcaccaagggtctgctgcaggatgtgacccagtatgccgagcagtacaagaacgacttcgcatccggcccgtacagcctggttcaggttggcggcaaggcttacggcctgccgcaggacaccggcccgctggtttacttctacaacaaggctgagttcgagaagctcggcatcaccgagattccgcagaccgccgatgagtttatcgccgctgccaagaccgctgccgccgctggcaagtacatcatgtcctaccagcctgatgaggccggcaacatgatctccggtctggctggcgcctccggtggttggtacaaggtgaagggcgactcctgggtcgtcaacaccgagaccgatggctccaaggcaaccgctgacttctaccagcagctgctcgacgccaaggcagccaccaccaacccgcgttgggatccgtccttcgatgcatccatcaaggatggctcgttgatcggtactgtggccgccgcttgggaagccccgctgttcatgacctcctccggtggcaccggctccggcgaatggcaggtcgctcagctcggtgactggttcggcaacgctggcaagaccggccctgacggtggttccgccgtggccgtgctgaagaactccaagcacccgaaggaagcaatggagttcctggattggttcaacacccaggttcctgatctggtttcccagggcctcgtgccggctgctaccactgaagacgctgagactccttccgagtggtccaccttcttcggtggtcaggacatcatgaaggaattcaagaccgctaacaacaacatgggtgacttcacctacatgcctggcttctccgcagtcgccgccaagatgaacgaaaccgccgccaaggccaccgatggctccggcaaggttgcagacatcttctccgacgcacagaccacctctgtggatacgctgaagaacttcggcctgtctgtttccgagctcgagatcaccaacctctgccccttcggcgaagtgttcaacgccacgcgctttgcctccgtgtatgcttggaatcgtaaaaggatctccaattgcgtcgctgactattccgttctgtataattccgcctccttttcgacgttcaagtgctatggagttagccccacgaagctcaatgacctgtgcttcaccaacgtttatgcggatagctttgtcatccggggtgacgaagttaggcaaattgcgcccggccaaaccggtaaaatcgctgattacaactataaactgcccgacgatttcaccggttgcgttatcgcctggaattccaacaatctcgattcgaaggtcggaggtaactataactatctgtatcgtctgttccgtaaatccaatctgaaaccctttgaacgggacatttccaccgaaatttatcaagccggatccaccccgtgtaacggggttgaaggtttcaactgctacttcccgctgcaatcgtacggattccagcccaccaatggagtgggatatcaaccgtaccgtgtcgtggtgctgagcttcgaactcctgcacgcgcccgccacggtgtgtggatgaagcatgc

SEQ ID NO: 20 - protein, 635 aa, Artificial Sequence
  GLBP-S1B-332-526 fusion protein
MVSRNKRIVAAFAAVAAMGMGLAGCGSDTAGDTKTTDDGGVVNITYMHRLPDSEGMTLVNDIVAKWNKQHPDIQVKATKFDGKASDMIKKLETDVKSGEAPDLAQVGYAELPEVFTKGLLQDVTQYAEQYKNDFASGPYSLVQVGGKAYGLPQDTGPLVYFYNKAEFEKLGITEIPQTADEFIAAAKTAAAAGKYIMSYQPDEAGNMISGLAGASGGWYKVKGDSWVVNTETDGSKATADFYQQLLDAKAATTNPRWDPSFDASIKDGSLIGTVAAAWEAPLFMTSSGGTGSGEWQVAQLGDWFGNAGKTGPDGGSAVAVLKNSKHPKEAMEFLDWFNTQVPDLVSQGLVPAATTEDAETPSEWSTFFGGQDIMKEFKTANNNMGDFTYMPGFSAVAAKMNETAAKATDGSGKVADIFSDAQTTSVDTLKNFGLSVSELEITNLCPFGEVFNATRFASVYAWNRKRISNCVADYSVLYNSASFSTFKCYGVSPTKLNDLCFTNVYADSFVIRGDEVRQIAPGQTGKIADYNYKLPDDFTGCVIAWNSNNLDSKVGGNYNYLYRLFRKSNLKPFERDISTEIYQAGSTPCNGVEGFNCYFPLQSYGFQPTNGVGYQPYRVVVLSFELLHAPATVCG

SEQ ID NO: 21 - DNA, 2368 bp, Artificial Sequence
  GLBP-S1B-332-526 N501Y fusion gene
catatgggcgatggcgaggcgaacgccacggttgacggcacgcacttcaacgtgcgtagcctgtggcagctctaccagttgctgagactgctcgtgtagcgtctcattaaggtgcggtgccccctggtcgggtatcgcgccggcgacctgaaaaccgataatgttggcaagtgcttgcaatttgcggtggacgattgcaagctaacgtcttggattgttgccgctatccaatatctcattaggcctaccggtggaccaaaagtacgttgctttgtaaggggagttaatgaaatgaacaaactcgcacaatcgagcatcgaaccggtttaatgctactcgcctcaacgggacgcgcggtaattgttagctaagttgacaataaaagaatgagggcatacattagtaatcagtcatcacactgagatgatgatttcactacgaaggagtagagatatggtatctcgcaataagcgcatcgtggctgcttttgccgcggtagcagcaatgggaatgggcttggccggttgcggcagcgacactgccggcgacacgaagaccaccgatgatggtggcgtggtcaacatcacctacatgcaccgtctgccggattccgagggcatgactctggtcaacgacatcgttgccaagtggaataagcagcatccggatattcaggtcaaggccaccaagttcgatggtaaggcctctgacatgatcaagaagcttgagaccgacgtcaagtccggcgaggctccggatctggctcaggtcggttacgccgagctgcctgaggtcttcaccaagggtctgctgcaggatgtgacccagtatgccgagcagtacaagaacgacttcgcatccggcccgtacagcctggttcaggttggcggcaaggcttacggcctgccgcaggacaccggcccgctggtttacttctacaacaaggctgagttcgagaagctcggcatcaccgagattccgcagaccgccgatgagtttatcgccgctgccaagaccgctgccgccgctggcaagtacatcatgtcctaccagcctgatgaggccggcaacatgatctccggtctggctggcgcctccggtggttggtacaaggtgaagggcgactcctgggtcgtcaacaccgagaccgatggctccaaggcaaccgctgacttctaccagcagctgctcgacgccaaggcagccaccaccaacccgcgttgggatccgtccttcgatgcatccatcaaggatggctcgttgatcggtactgtggccgccgcttgggaagccccgctgttcatgacctcctccggtggcaccggctccggcgaatggcaggtcgctcagctcggtgactggttcggcaacgctggcaagaccggccctgacggtggttccgccgtggccgtgctgaagaactccaagcacccgaaggaagcaatggagttcctggattggttcaacacccaggttcctgatctggtttcccagggcctcgtgccggctgctaccactgaagacgctgagactccttccgagtggtccaccttcttcggtggtcaggacatcatgaaggaattcaagaccgctaacaacaacatgggtgacttcacctacatgcctggcttctccgcagtcgccgccaagatgaacgaaaccgccgccaaggccaccgatggctccggcaaggttgcagacatcttctccgacgcacagaccacctctgtggatacgctgaagaacttcggcctgtctgtttccgagctcgagatcaccaacctctgccccttcggcgaagtgttcaacgccacgcgctttgcctccgtgtatgcttggaatcgtaaaaggatctccaattgcgtcgctgactattccgttctgtataattccgcctccttttcgacgttcaagtgctatggagttagccccacgaagctcaatgacctgtgcttcaccaacgtttatgcggatagctttgtcatccggggtgacgaagttaggcaaattgcgcccggccaaaccggtaaaatcgctgattacaactataaactgcccgacgatttcaccggttgcgttatcgcctggaattccaacaatctcgattcgaaggtcggaggtaactataactatctgtatcgtctgttccgtaaatccaatctgaaaccctttgaacgggacatttccaccgaaatttatcaagccggatccaccccgtgtaacggggttgaaggtttcaactgctacttcccgctgcaatcgtacggattccagcccacctacggagtgggatatcaaccgtaccgtgtcgtggtgctgagcttcgaactcctgcacgcgcccgccacggtgtgtggatgaagcatgc

SEQ ID NO: 22 - protein, 635 aa, Artificial Sequence
  GLBP-S1B-332-526 N501Y fusion protein
MVSRNKRIVAAFAAVAAMGMGLAGCGSDTAGDTKTTDDGGVVNITYMHRLPDSEGMTLVNDIVAKWNKQHPDIQVKATKFDGKASDMIKKLETDVKSGEAPDLAQVGYAELPEVFTKGLLQDVTQYAEQYKNDFASGPYSLVQVGGKAYGLPQDTGPLVYFYNKAEFEKLGITEIPQTADEFIAAAKTAAAAGKYIMSYQPDEAGNMISGLAGASGGWYKVKGDSWVVNTETDGSKATADFYQQLLDAKAATTNPRWDPSFDASIKDGSLIGTVAAAWEAPLFMTSSGGTGSGEWQVAQLGDWFGNAGKTGPDGGSAVAVLKNSKHPKEAMEFLDWFNTQVPDLVSQGLVPAATTEDAETPSEWSTFFGGQDIMKEFKTANNNMGDFTYMPGFSAVAAKMNETAAKATDGSGKVADIFSDAQTTSVDTLKNFGLSVSELEITNLCPFGEVFNATRFASVYAWNRKRISNCVADYSVLYNSASFSTFKCYGVSPTKLNDLCFTNVYADSFVIRGDEVRQIAPGQTGKIADYNYKLPDDFTGCVIAWNSNNLDSKVGGNYNYLYRLFRKSNLKPFERDISTEIYQAGSTPCNGVEGFNCYFPLQSYGFQPTYGVGYQPYRVVVLSFELLHAPATVCG

SEQ ID NO: 23 - protein, 9 aa, Artificial Sequence
  SARS-CoV-2 epitope peptide MBL037
GNYNYLYRL

SEQ ID NO: 24 - protein, 8 aa, Artificial Sequence
  SARS-CoV-2 epitope peptide MBL045
YNYLYRLF

SEQ ID NO: 25 - DNA, 783 bp, Artificial Sequence
  CD40L
atgatcgaaacctactcccagccgtccccgcgctccgtggccaccggcttgccggcctccatgaagatcttcatgtacctgctgaccgtgttcctgatcacccagatgatcggctccgtgctgttcgccgtgtacctgcaccgccgcttggacaaggtggaagaagaagtgaacctgcatgaagacttcgtgttcatcaagaagctgaagcgctgcaacaagggcgaaggctccctgtccctgctgaactgcgaagaaatgcgccgccagttcgaagacctggtgaaggacatcaccctgaacaaggaagaaaagaaggaaaactccttcgaaatgcagcgcggcgacgaagacccgcagatcgccgcccatgtggtgtccgaagccaactccaacgccgcctccgtgctgcagtgggccaagaagggctactacaccatgaagtccaacctggtgatgctggaaaacggcaagcagctgaccgtgaagcgcgaaggcctgtactacgtgtacacccaggtgaccttctgctccaaccgcgaaccgtcctcccagcgcccgttcatcgtgggcctgtggctgaagccgtcctccggctccgaacgcatcctgctgaaggccgccaacacccactcctcctcccagctgtgcgaacagcagtccgtgcacctgggtggcgtgttcgaactgcaggccggtgcctccgtgttcgtgaacgtgaccgaagcctcccaggtgatccaccgcgtgggcttctcctccttcggcctgctgaagctgtga

SEQ ID NO: 26 - DNA, 34 bp, Artificial Sequence; identical to SEQ ID NO: 15
  Primer for pTK2064-gltA-f

SEQ ID NO: 27 - DNA, 17 bp, Artificial Sequence
  Primer for pTK2064-gltA-SP-r
gtcgctgccgcaaccgg

SEQ ID NO: 28 - DNA, 37 bp, Artificial Sequence
  Primer for pTK2064-mCD40L-f
ggttgcggcagcgacatgatcgaaacctactcccagc

SEQ ID NO: 29 - DNA, 35 bp, Artificial Sequence
  Primer for pTK2064-mCD40L-r
agggcctcgtgcatatcacagcttcagcaggccga